European Patent Specification EP 4 025 612 B1, published October 29, 2025. Title: Binding Members. Applicant: Scancell Limited. The sequence listing filed with the application follows.

SEQUENCE LISTING (20 sequences)

SEQ ID NO: 1 - DNA, 34 bp, artificial sequence
  artificial sequence
attaagatctaagatggtgtccacttctcagctc

SEQ ID NO: 2 - DNA, 32 bp, artificial sequence
  artificial sequence
aattcgtacgtttgatttccagcttggtgcct

SEQ ID NO: 3 - DNA, 34 bp, artificial sequence
  artificial sequence
taataagcttaagatgagagtgctgattcttttg

SEQ ID NO: 4 - DNA, 29 bp, artificial sequence
  artificial sequence
agagcagcgctggagacggtgactgaggt

SEQ ID NO: 5 - protein, 124 aa, murine
DVQLQESGPDLVKPSQSLSLTCTVTGYSITSGYSWHWIRQFPGNKLEWVGYIHYRGNTNYNPSLKSRISITRDTYKNQLFLRLNSVTTEDTATYYCAQEPVRNYAMDYWGQGTSVTVSSATTTA

SEQ ID NO: 6 - DNA, 374 bp, murine
gatgtgcagcttcaggagtcaggacctgacctggtgaaaccttctcagtcactttcactcacctgcactgtcactggctactccatcaccagtggttatagctggcactggatccggcagtttccaggaaacaaactggaatgggtgggctacatacactaccgtggtaacactaactacaacccatctctcaaaagtcgaatctcaatcactcgagacacatacaagaaccagctcttcctgcggttgaattctgtgactactgaggacacagccacatattattgtgcacaagaacctgtgaggaactatgctatggactactggggtcaaggaacctcagtcaccgtctcctcagctacaacaacagcccc

SEQ ID NO: 7 - protein, 130 aa, murine
DVQLQESGPDLVKPSQSLSLTCTVTGYSITSGYSWHWIRQFPGNKLEWVGYIHYRGNTNYNPSLKSRISITRDTYKNQFFLQLNSVTTEDTATYYCAQEPVRNYAMDYWGQGTSVTVSSATTTAPSIYPL

SEQ ID NO: 8 - DNA, 390 bp, murine
gatgtgcagcttcaggagtcaggacctgacctggtgaaaccttctcagtcactttcactcacctgcactgtcactggctactccatcaccagtggttatagctggcactggatccggcagtttccaggaaacaaactggaatgggtgggctacatacactaccgtggtaacactaactacaacccatctctcaaaagtcgaatctcaatcactcgagacacatacaagaaccagttcttcctgcagttgaattctgtgactactgaggacacagccacatattattgtgcacaagaacctgtgaggaactatgctatggactactggggtcaaggaacctcagtcaccgtctcctcagctacaacaacagccccatcaatctatccactg

SEQ ID NO: 9 - protein, 120 aa, murine
AVQLQESGPDLVKPSQSLSLTCTVTGYSITSGYSWHWIRQFPGNKLEWVGYIHYRGNTNYNPSLKSRVSITRDTYKNQFFLQLNSLTTEDTATYYCAQEPVRNYAMDFWGQGTSVTVSSA

SEQ ID NO: 10 - DNA, 360 bp, murine
gctgtgcaacttcaggagtcaggacctgacctggtgaaaccttctcagtcactttcactcacctgtactgtcactggctactccatcaccagtggttatagctggcactggatccggcagtttccaggaaacaaactggaatgggtgggctacatacactaccgtggtaacactaattacaacccatctctcaaaagtcgagtctcaatcactcgagacacatacaagaaccagttcttcctacagttaaattctctgactactgaggacacagccacatattattgtgcacaagaacctgtgaggaactatgctatggacttttggggtcaaggaacctcagtcaccgtctccagcgct

SEQ ID NO: 11 - protein, 103 aa, murine
DIVMSQSPATLSVTPGDRVSLSCRASQSIGDDLHWYQQKSHESPRLLIKYVSQSISGIPSRFSGSGSGSYFTLTINSVEPEDVGVYYCQNGHGFPPTFGGGTK

SEQ ID NO: 12 - DNA, 309 bp, murine
gacattgtgatgagtcagtctccagccaccctgtctgtgactccaggagatagagtctctctttcctgcagggccagccagagtattggcgacgacttacactggtatcaacaaaaatcacatgagtctccaaggcttctcatcaaatatgtttcccaatccatctctgggatcccctccaggttcagtggcagtggatcagggtcatatttcactctcactatcaacagtgtggaacctgaagatgttggagtatattactgtcaaaatggtcacggctttcctccgacgttcggtggaggcaccaag

SEQ ID NO: 13 - protein, 103 aa, murine
DIVMSQSPATLSVTPGDRVSLSCRASQSISDDLHWYQQKSHESPRLLIKYVSQYISGIPSRFSGSGSGSDFTLTIKSVEPEDVGVYYCQNGYSFPPTFGGGTK

SEQ ID NO: 14 - DNA, 309 bp, murine
gacattgtgatgagtcagtctccagccaccctgtctgtgactccaggagatagagtctctctttcctgcagggccagccagagtattagcgacgacttacactggtatcaacaaaaatcacatgagtctccaaggcttctcatcaaatatgtttcccaatacatctctgggatcccctccaggttcagtggcagtggatcagggtcagatttcactctcactatcaagagtgtggaacctgaagatgttggagtatattactgtcaaaatggttacagctttcctccgacgttcggtggaggcaccaag

SEQ ID NO: 15 - protein, 109 aa, murine
DIVMTQSPDTLSVTPGDRVSLSCRASQSISDDLHWYQQKSHESPRLLIKYVSQSISGIPSRFSGSGSRSDFTLTINSVEPEDVGLYYCQNGHGFPPTFGGGTKLEIKRT

SEQ ID NO: 16 - DNA, 327 bp, murine
gacattgtgatgactcagtctccagacaccctgtctgtgactccaggagatagagtctctctttcctgcagggccagccagagtattagcgacgacttacactggtatcaacaaaaatcacatgagtctccaagacttctcatcaaatatgtttctcaatccatctctgggatcccctccaggttcagtggcagtggatcaagatcagatttcactctcactatcaacagtgtggaacctgaagatgttggactatattactgtcaaaatggtcacggctttcctccgacgttcggtggaggcaccaagctggaaatcaaacgtacg

SEQ ID NO: 17 - DNA, 1347 bp, artificial sequence
  Human/mouse chimeric sequence
gctgtgcaacttcaggagtcaggacctgacctggtgaaaccttctcagtcactttcactcacctgtactgtcactggctactccatcaccagtggttatagctggcactggatccggcagtttccaggaaacaaactggaatgggtgggctacatacactaccgtggtaacactaattacaacccatctctcaaaagtcgagtctcaatcactcgagacacatacaagaaccagttcttcctacagttaaattctctgactactgaggacacagccacatattattgtgcacaagaacctgtgaggaactatgctatggacttttggggtcaaggaacctcagtcaccgtctccagcgcttccaccaagggcccatcggtcttccccctggcaccctcctccaagagcacctctgggggcacagcggccctgggctgcctggtcaaggactacttccccgaaccggtgacggtgtcgtggaactcaggcgccctgaccagcggcgtgcacaccttcccggctgtcctacagtcctcaggactctactccctcagcagcgtggtgaccgtgccctccagcagcttgggcacccagacctacatctgcaacgtgaatcacaagcccagcaacaccaaggtggacaagaaagttgagcccaaatcttgtgacaaaactcacacatgcccaccgtgcccagcacctgaactcctggggggaccgtcagtcttcctcttccccccaaaacccaaggacaccctcatgatctcccggacccctgaggtcacatgcgtggtggtggacgtgagccacgaagaccctgaggtcaagttcaactggtacgtggacggcgtggaggtgcataatgccaagacaaagccgcgggaggagcagtacaacagcacgtaccgtgtggtcagcgtcctcaccgtcctgcaccaggactggctgaatggcaaggagtacaagtgcaaggtctccaacaaagccctcccagcccccatcgagaaaaccatctccaaagccaaagggcagccccgagaaccacaggtgtacaccctgcccccatcccgggatgagctgaccaagaaccaggtcagcctgacctgcctggtcaaaggcttctatcccagcgacatcgccgtggagtgggagagcaatgggcagccggagaacaactacaagaccacgcctcccgtgctggactccgacggctccttcttcctctacagcaagctcaccgtggacaagagcaggtggcagcaggggaacgtcttctcatgctccgtgatgcatgaggctctgcacaaccactacacgcagaagagcctctccctgtctccgggtaaa

SEQ ID NO: 18 - protein, 449 aa, artificial sequence
  Human/mouse chimeric sequence
AVQLQESGPDLVKPSQSLSLTCTVTGYSITSGYSWHWIRQFPGNKLEWVGYIHYRGNTNYNPSLKSRVSITRDTYKNQFFLQLNSLTTEDTATYYCAQEPVRNYAMDFWGQGTSVTVSSASTKGPSVFPLAPSSKSTSGGTAALGCLVKDYFPEPVTVSWNSGALTSGVHTFPAVLQSSGLYSLSSVVTVPSSSLGTQTYICNVNHKPSNTKVDKKVEPKSCDKTHTCPPCPAPELLGGPSVFLFPPKPKDTLMISRTPEVTCVVVDVSHEDPEVKFNWYVDGVEVHNAKTKPREEQYNSTYRVVSVLTVLHQDWLNGKEYKCKVSNKALPAPIEKTISKAKGQPREPQVYTLPPSRDELTKNQVSLTCLVKGFYPSDIAVEWESNGQPENNYKTTPPVLDSDGSFFLYSKLTVDKSRWQQGNVFSCSVMHEALHNHYTQKSLSLSPGK

SEQ ID NO: 19 - DNA, 642 bp, artificial sequence
  Human/mouse chimeric sequence
gacattgtgatgactcagtctccagacaccctgtctgtgactccaggagatagagtctctctttcctgcagggccagccagagtattagcgacgacttacactggtatcaacaaaaatcacatgagtctccaagacttctcatcaaatatgtttctcaatccatctctgggatcccctccaggttcagtggcagtggatcaagatcagatttcactctcactatcaacagtgtggaacctgaagatgttggactatattactgtcaaaatggtcacggctttcctccgacgttcggtggaggcaccaagctggaaatcaaacgtacggtagcggccccatctgtcttcatcttcccgccatctgatgagcagttgaaatctggaactgcctctgttgtgtgcctgctgaataacttctatcccagagaggccaaagtacagtggaaggtggataacgccctccaatcgggtaactcccaggagagtgtcacagagcaggacagcaaggacagcacctacagcctcagcagcaccctgacgctgagcaaagcagactacgagaaacacaaagtctacgcctgcgaagtcacccatcagggcctgagctcgcccgtcacaaagagcttcaacaggggagagtgt

SEQ ID NO: 20 - protein, 214 aa, artificial sequence
  Human/mouse chimeric sequence
DIVMTQSPDTLSVTPGDRVSLSCRASQSISDDLHWYQQKSHESPRLLIKYVSQSISGIPSRFSGSGSRSDFTLTINSVEPEDVGLYYCQNGHGFPPTFGGGTKLEIKRTVAAPSVFIFPPSDEQLKSGTASVVCLLNNFYPREAKVQWKVDNALQSGNSQESVTEQDSKDSTYSLSSTLTLSKADYEKHKVYACEVTHQGLSSPVTKSFNRGEC